European Patent Application EP 4 357 358 A1, published April 24, 2024. Title: GLUCAGON ANALOG AND MEDICAL USE THEREOF. Applicant: BEIJING TUO JIE BIOPHARMACEUTICAL CO., LTD. Application PCT/CN2022/099357. The sequence listing filed with the application follows.

SEQUENCE LISTING (52 sequences)

SEQ ID NO: 1 - protein, 29 aa, Artificial Sequence
  Synthesized compound
  MOD_RES (13)..(13): Xaa is Aib
HSQGTFTSDYSKXLDSRRAQDFVQWLMNT

SEQ ID NO: 2 - protein, 29 aa, Artificial Sequence
  Synthesized compound
  MOD_RES (16)..(16): Xaa is alpha-methyl-Ser
HSQGTFTSDYSKYLDXRRAQDFVQWLMNT

SEQ ID NO: 3 - protein, 29 aa, Artificial Sequence
  Synthesized compound
  MOD_RES (17)..(17): Xaa is Aib
HSQGTFTSDYSKYLDSXRAQDFVQWLMNT

SEQ ID NO: 4 - protein, 29 aa, Artificial Sequence
  Synthesized compound
  MOD_RES (18)..(18): Xaa is Aib
HSQGTFTSDYSKYLDSRXAQDFVQWLMNT

SEQ ID NO: 5 - protein, 29 aa, Artificial Sequence
  Synthesized compound
  MOD_RES (24)..(24): Xaa is alpha-methyl-Ser
HSQGTFTSDYSKYLDSRRAQDFVXWLMNT

SEQ ID NO: 6 - protein, 29 aa, Artificial Sequence
  Synthesized compound
  MOD_RES (18)..(18): Xaa is Aib
HSQGTFTSDYSKYLESRXAEDFVQWLMNT

SEQ ID NO: 7 - protein, 29 aa, Artificial Sequence
  Synthesized compound
  MOD_RES (18)..(18): Xaa is Aib
HSQGTFTSDYSKYLESRXAEDFVQWLLET

SEQ ID NO: 8 - protein, 29 aa, Artificial Sequence
  Synthesized compound
  MOD_RES (18)..(18): Xaa is Aib
HSQGTFTSDYSKYLESRXAQEFVEWLMNT

SEQ ID NO: 9 - protein, 29 aa, Artificial Sequence
  Synthesized compound
  MOD_RES (18)..(18): Xaa is Aib
HSQGTFTSDYSKYLESRXAQEFVEWLLST

SEQ ID NO: 10 - protein, 29 aa, Artificial Sequence
  Synthesized compound
  MOD_RES (18)..(18): Xaa is Aib
HSQGTFTSDYSKYLESRXAQEFVSWLLET

SEQ ID NO: 11 - protein, 29 aa, Artificial Sequence
  Synthesized compound
  MOD_RES (18)..(18): Xaa is Aib
HSQGTFTSDYSKYLDSRXAEEFVSWLLST

SEQ ID NO: 12 - protein, 29 aa, Artificial Sequence
  Synthesized compound
  MOD_RES (18)..(18): Xaa is Aib
HSQGTFTSDYSKYLDTRXAEEFVSWLSET

SEQ ID NO: 13 - protein, 29 aa, Artificial Sequence
  Synthesized compound
  MOD_RES (17)..(17): Xaa is Aib
HSQGTFTSDYSKYLESXRAQEFVQWLMNT

SEQ ID NO: 14 - protein, 29 aa, Artificial Sequence
  Synthesized compound
  MOD_RES (17)..(17): Xaa is Aib
HSQGTFTSDYSKYLDSXRAQDFVQWLLST

SEQ ID NO: 15 - protein, 29 aa, Artificial Sequence
  Synthesized compound
  MOD_RES (17)..(17): Xaa is Aib
HSQGTFTSDYSKYLDSXRAQDFVQWLEST

SEQ ID NO: 16 - protein, 29 aa, Artificial Sequence
  Synthesized compound
  MOD_RES (17)..(17): Xaa is Aib
HSQGTFTSDYSKYLDSXRAQDFVQWLLET

SEQ ID NO: 17 - protein, 29 aa, Artificial Sequence
  Synthesized compound
  MOD_RES (17)..(17): Xaa is Aib
HSQGTFTSDYSKYLESXRAQEFVQWLLST

SEQ ID NO: 18 - protein, 29 aa, Artificial Sequence
  Synthesized compound
  MOD_RES (17)..(17): Xaa is Aib
HSQGTFTSDYSKYLESXRAQEFVQWLEST

SEQ ID NO: 19 - protein, 29 aa, Artificial Sequence
  Synthesized compound
  MOD_RES (17)..(17): Xaa is Aib
HSQGTFTSDYSKYLESXRAQEFVQWLLET

SEQ ID NO: 20 - protein, 29 aa, Artificial Sequence
  Synthesized compound
  MOD_RES (17)..(17): Xaa is Aib
HSQGTFTSDYSKYLESXRAQEFVEWLLST

SEQ ID NO: 21 - protein, 29 aa, Artificial Sequence
  Synthesized compound
  MOD_RES (17)..(17): Xaa is Aib
HSQGTFTSDYSKYLESXRAQEFVEWLEST

SEQ ID NO: 22 - protein, 29 aa, Artificial Sequence
  Synthesized compound
  MOD_RES (17)..(17): Xaa is Aib
HSQGTFTSDYSKYLESXRAQEFVEWLLET

SEQ ID NO: 23 - protein, 29 aa, Artificial Sequence
  Synthesized compound
  MOD_RES (18)..(18): Xaa is Aib
HSQGTFTSDYSKYLESRXAQEFVEWLEST

SEQ ID NO: 24 - protein, 29 aa, Artificial Sequence
  Synthesized compound
  MOD_RES (18)..(18): Xaa is Aib
HSQGTFTSDYSKYLESRXAQEFVEWLLET

SEQ ID NO: 25 - protein, 29 aa, Artificial Sequence
  Synthesized compound
  MOD_RES (18)..(18): Xaa is Aib
HSQGTFTSDYSKYLESKXAQEFVEWLEST

SEQ ID NO: 26 - protein, 29 aa, Artificial Sequence
  Synthesized compound
  MOD_RES (18)..(18): Xaa is Aib
HSQGTFTSDYSKYLESEXAQEFVEWLEST

SEQ ID NO: 27 - protein, 29 aa, Artificial Sequence
  Synthesized compound
  MOD_RES (17)..(17): Xaa is Aib
HSQGTFTSDYSKYLESXRAQDFVQWLLST

SEQ ID NO: 28 - protein, 29 aa, Artificial Sequence
  Synthesized compound
  MOD_RES (17)..(17): Xaa is Aib
HSQGTFTSDYSKYLESXRAQDFVQWLEST

SEQ ID NO: 29 - protein, 29 aa, Artificial Sequence
  Synthesized compound
  MOD_RES (17)..(17): Xaa is Aib
HSQGTFTSDYSKYLESXRAQDFVQWLLET

SEQ ID NO: 30 - protein, 29 aa, Artificial Sequence
  Synthesized compound
  MOD_RES (17)..(17): Xaa is Aib
HSQGTFTSDYSKYLESXRAQDFVQWLEET

SEQ ID NO: 31 - protein, 29 aa, Artificial Sequence
  Synthesized compound
  MOD_RES (17)..(17): Xaa is Aib
HSQGTFTSDYSKYLESXRAQEFVQWLEET

SEQ ID NO: 32 - protein, 29 aa, Artificial Sequence
  Synthesized compound
  MOD_RES (17)..(17): Xaa is Aib
HSQGTFTSDYSKYLESXRAQDFVEWLLST

SEQ ID NO: 33 - protein, 29 aa, Artificial Sequence
  Synthesized compound
  MOD_RES (17)..(17): Xaa is Aib
HSQGTFTSDYSKYLESXRAQDFVEWLEST

SEQ ID NO: 34 - protein, 29 aa, Artificial Sequence
  Synthesized compound
  MOD_RES (17)..(17): Xaa is Aib
HSQGTFTSDYSKYLESXRAQDFVEWLLET

SEQ ID NO: 35 - protein, 29 aa, Artificial Sequence
  Synthesized compound
  MOD_RES (17)..(17): Xaa is Aib
HSQGTFTSDYSKYLESXRAQDFVEWLEET

SEQ ID NO: 36 - protein, 29 aa, Artificial Sequence
  Synthesized compound
  MOD_RES (17)..(17): Xaa is Aib
HSQGTFTSDYSKYLESXRAQEFVEWLEET

SEQ ID NO: 37 - protein, 29 aa, Artificial Sequence
  Synthesized compound
  MOD_RES (17)..(17): Xaa is Aib
HSQGTFTSDYSKYLESXRAKDFVEWLEST

SEQ ID NO: 38 - protein, 28 aa, Artificial Sequence
  Synthesized compound
  MOD_RES (17)..(17): Xaa is Aib
HSQGTFTSDYSKYLESXRAEDFVRWLES

SEQ ID NO: 39 - protein, 29 aa, Artificial Sequence
  Synthesized compound
  MOD_RES (17)..(17): Xaa is Aib
HSQGTFTSDYSKYLDTXRAQEFVQWLEST

SEQ ID NO: 40 - protein, 29 aa, Artificial Sequence
  Synthesized compound
  MOD_RES (17)..(17): Xaa is Aib
HSQGTFTSDYSKYLDLXRAQEFVQWLEST

SEQ ID NO: 41 - protein, 29 aa, Artificial Sequence
  Synthesized compound
  MOD_RES (17)..(17): Xaa is Aib
HSQGTFTSDYSKYLDVXRAQEFVQWLEST

SEQ ID NO: 42 - protein, 29 aa, Artificial Sequence
  Synthesized compound
  MOD_RES (17)..(17): Xaa is Aib
HSQGTFTSDYSKYLDIXRAQEFVQWLEST

SEQ ID NO: 43 - protein, 29 aa, Artificial Sequence
  Synthesized compound
  MOD_RES (17)..(17): Xaa is Aib
HSHGTFTSDYSKYLDLXRAQEFVQWLEST

SEQ ID NO: 44 - protein, 29 aa, Artificial Sequence
  Synthesized compound
  MOD_RES (17)..(17): Xaa is Aib
HSQGTFTSDYSKYLDLXRAEDFVRWLEST

SEQ ID NO: 45 - protein, 29 aa, Artificial Sequence
  Synthesized compound
  MOD_RES (17)..(17): Xaa is Aib
HSQGTFTSDYSKYLDLXRAEDFVQWLEST

SEQ ID NO: 46 - protein, 29 aa, Artificial Sequence
  Synthesized compound
  MOD_RES (17)..(17): Xaa is Aib
HSHGTFTSDYSKYLDLXRAEEFVQWLEST

SEQ ID NO: 47 - protein, 29 aa, Artificial Sequence
  Synthesized compound
  MOD_RES (17)..(17): Xaa is Aib
HSHGTFTSDYSKYLDLXRAQEFVEWLEST

SEQ ID NO: 48 - protein, 29 aa, Artificial Sequence
  Synthesized compound
  MOD_RES (17)..(17): Xaa is Aib
HSQGTFTSDYSKYLDLXRAEEFVRWLEST

SEQ ID NO: 49 - protein, 29 aa, Artificial Sequence
  Synthesized compound
  MOD_RES (17)..(17): Xaa is Aib
HSQGTFTSDYSKYLDLXRAEEFVQWLEST

SEQ ID NO: 50 - protein, 29 aa, Artificial Sequence
  Synthesized compound
  SITE (3)..(3): Xaa may be any natural amino acid residue or unnatural amino acid residue
  SITE (15)..(15): Xaa may be any natural amino acid residue or unnatural amino acid residue
  SITE (16)..(16): Xaa may be any natural amino acid residue or unnatural amino acid residue
  MOD_RES (17)..(17): Xaa is Aib
  SITE (20)..(20): Xaa may be any natural amino acid residue or unnatural amino acid residue
  SITE (21)..(21): Xaa may be any natural amino acid residue or unnatural amino acid residue
  SITE (24)..(24): Xaa may be any natural amino acid residue or unnatural amino acid residue
  SITE (27)..(27): Xaa may be any natural amino acid residue or unnatural amino acid residue
  SITE (28)..(28): Xaa may be any natural amino acid residue or unnatural amino acid residue
HSXGTFTSDYSKYLXXXRAXXFVXWLXXT

SEQ ID NO: 51 - protein, 29 aa, Homo sapiens
HSQGTFTSDYSKYLDSRRAQDFVQWLMNT

SEQ ID NO: 52 - protein, 29 aa, Artificial Sequence
  Synthesized compound
  MOD_RES (16)..(16): Xaa is Aib
HSQGTFTSDYSKYLDXARAEEFVKWLEST